European Patent Specification EP 3 468 999 B1, published January 10, 2024. Title: Anti-GITR Antibodies and Uses Thereof. Applicant: Regeneron Pharmaceuticals, Inc. The sequence listing filed with the application follows.

SEQUENCE LISTING (413 sequences)

SEQ ID NO: 1 - DNA, 369 bp, Artificial Sequence
  synthetic
caggtgcagctggtggagtctgggggaggcgtggtccagcctgggaggtccctgagactctcctgtgcagcgtctggattcaccttcagtagttatggcatggactgggtccgccaggctccaggcaaggggctggagtgggtggcagttatatggtatcctggaagtaataaatactatgcagactccgtgaagggccgattcaccgtctccagagacaattccaagaacacgctgtatctgcaaatgaacagcctgagagccgaggacacggctgtgtattactgtgcgagagacggagaactgggactggactactactccggcatggacgtctggggccaagggaccacggtcaccgtctcctca

SEQ ID NO: 2 - protein, 123 aa, Artificial Sequence
  synthetic
QVQLVESGGGVVQPGRSLRLSCAASGFTFSSYGMDWVRQAPGKGLEWVAVIWYPGSNKYYADSVKGRFTVSRDNSKNTLYLQMNSLRAEDTAVYYCARDGELGLDYYSGMDVWGQGTTVTVSS

SEQ ID NO: 3 - DNA, 24 bp, Artificial Sequence
  synthetic
ggattcaccttcagtagttatggc

SEQ ID NO: 4 - protein, 8 aa, Artificial Sequence
  synthetic
GFTFSSYG

SEQ ID NO: 5 - DNA, 24 bp, Artificial Sequence
  synthetic
atatggtatcctggaagtaataaa

SEQ ID NO: 6 - protein, 8 aa, Artificial Sequence
  synthetic
IWYPGSNK

SEQ ID NO: 7 - DNA, 48 bp, Artificial Sequence
  synthetic
gcgagagacggagaactgggactggactactactccggcatggacgtc

SEQ ID NO: 8 - protein, 16 aa, Artificial Sequence
  synthetic
ARDGELGLDYYSGMDV

SEQ ID NO: 9 - DNA, 321 bp, Artificial Sequence
  synthetic
gacatccagatgacccagtctccatcctccctgtctgcatctgtaggagacagagtcaccatcacttgccgggcaagtcagggcattagaaatgatttaaactggtatcagcagaaaccagggaaagcccctaagcgcctgatcaatggtgcatccagtttgcaaagtggggtcccatcaaggttcagcggcagtggatctgggacagaattcactctcacaatcagcagcctgcagcctgaagattttgcaacttattactgtctacaacttaatagttaccctcggacgttcggccaagggaccaaggtggaaatcaaa

SEQ ID NO: 10 - protein, 107 aa, Artificial Sequence
  synthetic
DIQMTQSPSSLSASVGDRVTITCRASQGIRNDLNWYQQKPGKAPKRLINGASSLQSGVPSRFSGSGSGTEFTLTISSLQPEDFATYYCLQLNSYPRTFGQGTKVEIK

SEQ ID NO: 11 - DNA, 18 bp, Artificial Sequence
  synthetic
cagggcattagaaatgat

SEQ ID NO: 12 - protein, 6 aa, Artificial Sequence
  synthetic
QGIRND

SEQ ID NO: 13 - DNA, 9 bp, Artificial Sequence
  synthetic
ggtgcatcc

SEQ ID NO: 14 - protein, 3 aa, Artificial Sequence
  synthetic
GAS

SEQ ID NO: 15 - DNA, 27 bp, Artificial Sequence
  synthetic
ctacaacttaatagttaccctcggacg

SEQ ID NO: 16 - protein, 9 aa, Artificial Sequence
  synthetic
LQLNSYPRT

SEQ ID NO: 17 - DNA, 369 bp, Artificial Sequence
  synthetic
caggtgcagctggtggagtctgggggaggcgtggtccagcctgggaggtccctgagactctcctgtgcagcgtctggattcaccttcagcaactatggcatgcactgggtccgccaggctccaggcaaggggctggagtgggtggcagttatatggtatcctggaagtaataagttctatacagactccgtggagggccgattcaccatctccagagacaattccaagaacacggtatatctacaaatggacagcctgagagccgaagacacggctgtgtattactgtgcgagagggggggcactgggggtagactattactacggtatggacgtctggggccaagggaccacggtcaccgtctcctca

SEQ ID NO: 18 - protein, 123 aa, Artificial Sequence
  synthetic
QVQLVESGGGVVQPGRSLRLSCAASGFTFSNYGMHWVRQAPGKGLEWVAVIWYPGSNKFYTDSVEGRFTISRDNSKNTVYLQMDSLRAEDTAVYYCARGGALGVDYYYGMDVWGQGTTVTVSS

SEQ ID NO: 19 - DNA, 24 bp, Artificial Sequence
  synthetic
ggattcaccttcagcaactatggc

SEQ ID NO: 20 - protein, 8 aa, Artificial Sequence
  synthetic
GFTFSNYG

SEQ ID NO: 21 - DNA, 24 bp, Artificial Sequence
  synthetic
atatggtatcctggaagtaataag

SEQ ID NO: 22 - protein, 8 aa, Artificial Sequence
  synthetic
IWYPGSNK

SEQ ID NO: 23 - DNA, 48 bp, Artificial Sequence
  synthetic
gcgagagggggggcactgggggtagactattactacggtatggacgtc

SEQ ID NO: 24 - protein, 16 aa, Artificial Sequence
  synthetic
ARGGALGVDYYYGMDV

SEQ ID NO: 25 - DNA, 321 bp, Artificial Sequence
  synthetic
gccatccagatgacccagtctccatcctccctgtctgcatctgtaggagacagagtcaccctcacttgccgggcaagtcagggcattagaaatgatttaggctggtatcagcagaaaccagggaaagcccctaatttcctgatctattctgcatccagtttacaaagtggggtcccatcaaggttcagcggcagtggatctggcacagatttcactctcaccatcagcagcctacagcctgaggattttgcaacttattactgtctacaaaattacaattacccgtggacgttcggccaagggaccaaggtggaaatcaaa

SEQ ID NO: 26 - protein, 107 aa, Artificial Sequence
  synthetic
AIQMTQSPSSLSASVGDRVTLTCRASQGIRNDLGWYQQKPGKAPNFLIYSASSLQSGVPSRFSGSGSGTDFTLTISSLQPEDFATYYCLQNYNYPWTFGQGTKVEIK

SEQ ID NO: 27 - DNA, 18 bp, Artificial Sequence
  synthetic
cagggcattagaaatgat

SEQ ID NO: 28 - protein, 6 aa, Artificial Sequence
  synthetic
QGIRND

SEQ ID NO: 29 - DNA, 9 bp, Artificial Sequence
  synthetic
tctgcatcc

SEQ ID NO: 30 - protein, 3 aa, Artificial Sequence
  synthetic
SAS

SEQ ID NO: 31 - DNA, 27 bp, Artificial Sequence
  synthetic
ctacaaaattacaattacccgtggacg

SEQ ID NO: 32 - protein, 9 aa, Artificial Sequence
  synthetic
LQNYNYPWT

SEQ ID NO: 33 - DNA, 372 bp, Artificial Sequence
  synthetic
caggtgcagctggtggagtctgggggaggcgtggtccagcctgggaggtccctgagactctcctgtgttgcgtctggattcaccttcagtgactatggcatgcactgggtccgccaggctccaggcaaggggctagagtgggtggcagttatatggtatgaaggaagtaataaatattatgcagactccgtgacgggccgattcaccatctccagagacaattccaagaacacgctgtttctgcaaatgaacagtctgaaagccgaagacacggctgagtattattgtgcgaaagatggggggcagctcgcctaccagtattactacggcatggacgtctggggccaagggaccacggtcaccgtctcctca

SEQ ID NO: 34 - protein, 124 aa, Artificial Sequence
  synthetic
QVQLVESGGGVVQPGRSLRLSCVASGFTFSDYGMHWVRQAPGKGLEWVAVIWYEGSNKYYADSVTGRFTISRDNSKNTLFLQMNSLKAEDTAEYYCAKDGGQLAYQYYYGMDVWGQGTTVTVSS

SEQ ID NO: 35 - DNA, 24 bp, Artificial Sequence
  synthetic
ggattcaccttcagtgactatggc

SEQ ID NO: 36 - protein, 8 aa, Artificial Sequence
  synthetic
GFTFSDYG

SEQ ID NO: 37 - DNA, 24 bp, Artificial Sequence
  synthetic
atatggtatgaaggaagtaataaa

SEQ ID NO: 38 - protein, 8 aa, Artificial Sequence
  synthetic
IWYEGSNK

SEQ ID NO: 39 - DNA, 51 bp, Artificial Sequence
  synthetic
gcgaaagatggggggcagctcgcctaccagtattactacggcatggacgtc

SEQ ID NO: 40 - protein, 17 aa, Artificial Sequence
  synthetic
AKDGGQLAYQYYYGMDV

SEQ ID NO: 41 - DNA, 321 bp, Artificial Sequence
  synthetic
gccatccagatgacccagtctccatcctccctgtctgcatctgtaggagacagagtcaccctcacttgccgggcaagtcagggcattagaaatgatttaggctggtatcagcagaaaccaggaaaagcccctaagagcctgatctatgctgcttccaatttacaaagtggagtcccttcaaggttcagcggcagtggatctggcacagatttcactctcaccatcagcagcctgcagcctgaggattctgcaacttattactgtctacaagactacaattaccctcggacgttcggccaagggaccaaggtggaaatcaaa

SEQ ID NO: 42 - protein, 107 aa, Artificial Sequence
  synthetic
AIQMTQSPSSLSASVGDRVTLTCRASQGIRNDLGWYQQKPGKAPKSLIYAASNLQSGVPSRFSGSGSGTDFTLTISSLQPEDSATYYCLQDYNYPRTFGQGTKVEIK

SEQ ID NO: 43 - DNA, 18 bp, Artificial Sequence
  synthetic
cagggcattagaaatgat

SEQ ID NO: 44 - protein, 6 aa, Artificial Sequence
  synthetic
QGIRND

SEQ ID NO: 45 - DNA, 9 bp, Artificial Sequence
  synthetic
gctgcttcc

SEQ ID NO: 46 - protein, 3 aa, Artificial Sequence
  synthetic
AAS

SEQ ID NO: 47 - DNA, 27 bp, Artificial Sequence
  synthetic
ctacaagactacaattaccctcggacg

SEQ ID NO: 48 - protein, 9 aa, Artificial Sequence
  synthetic
LQDYNYPRT

SEQ ID NO: 49 - DNA, 369 bp, Artificial Sequence
  synthetic
caggtgcagctggtggagtctgggggaggcgtggtccagcctgggaggtccctgagactctcctgtgcagcgtctggattcaacttcaggagctatggcatgcactgggtccgccaggctccaggcaaggggctggagtgggtggcagttatatggtatgatggaagtaataaatattatgcagactccgtgaagggccgattcaccatctccagagacagttccagggacacgctgtttctgcaaatgaacagcctgagagccggggacacggctgtgtattactgtgcgagaggaggtatgttgggacgggactactactacggtatggacgtctggggccaagggaccacggtcaccgtctcctca

SEQ ID NO: 50 - protein, 123 aa, Artificial Sequence
  synthetic
QVQLVESGGGVVQPGRSLRLSCAASGFNFRSYGMHWVRQAPGKGLEWVAVIWYDGSNKYYADSVKGRFTISRDSSRDTLFLQMNSLRAGDTAVYYCARGGMLGRDYYYGMDVWGQGTTVTVSS

SEQ ID NO: 51 - DNA, 24 bp, Artificial Sequence
  synthetic
ggattcaacttcaggagctatggc

SEQ ID NO: 52 - protein, 8 aa, Artificial Sequence
  synthetic
GFNFRSYG

SEQ ID NO: 53 - DNA, 24 bp, Artificial Sequence
  synthetic
atatggtatgatggaagtaataaa

SEQ ID NO: 54 - protein, 8 aa, Artificial Sequence
  synthetic
IWYDGSNK

SEQ ID NO: 55 - DNA, 48 bp, Artificial Sequence
  synthetic
gcgagaggaggtatgttgggacgggactactactacggtatggacgtc

SEQ ID NO: 56 - protein, 16 aa, Artificial Sequence
  synthetic
ARGGMLGRDYYYGMDV

SEQ ID NO: 57 - DNA, 321 bp, Artificial Sequence
  synthetic
gacatccagatgacccagtctccatcctccctgtctgcatctgtaggagacagagtcaccatcacttgccgggcaagtcagggcattagaaatgatttaggctggtatcagcagaaaccagggaaagcccctaagcgcctgatctatgctgcatccagtttgcaaagtggggtcccatcaaggttcagcggcagtggatctgggacagaattcactctcacaatcagcagcctgcagcctgaagattttgcaacttattactgtctacaacataatagttacccgaacacttttggccaggggaccaagctggagatcaaa

SEQ ID NO: 58 - protein, 107 aa, Artificial Sequence
  synthetic
DIQMTQSPSSLSASVGDRVTITCRASQGIRNDLGWYQQKPGKAPKRLIYAASSLQSGVPSRFSGSGSGTEFTLTISSLQPEDFATYYCLQHNSYPNTFGQGTKLEIK

SEQ ID NO: 59 - DNA, 18 bp, Artificial Sequence
  synthetic
cagggcattagaaatgat

SEQ ID NO: 60 - protein, 6 aa, Artificial Sequence
  synthetic
QGIRND

SEQ ID NO: 61 - DNA, 9 bp, Artificial Sequence
  synthetic
gctgcatcc

SEQ ID NO: 62 - protein, 3 aa, Artificial Sequence
  synthetic
AAS

SEQ ID NO: 63 - DNA, 27 bp, Artificial Sequence
  synthetic
ctacaacataatagttacccgaacact

SEQ ID NO: 64 - protein, 9 aa, Artificial Sequence
  synthetic
LQHNSYPNT

SEQ ID NO: 65 - DNA, 369 bp, Artificial Sequence
  synthetic
caggtgcagctggtggagtctgggggaggcgcggtccagcctgggacgtccctgagactctcctgcgcggcgtctggattcaccttcagtagttttggcatgcactgggtccgccaggctccaggcaaggggctggagtgggtgtcagttatatggtatgaggggagtaataaatattatgcagattcagtgaagggccgattcaccatctccagagacaattccagaaacacgctgagtctgcaaatggacagcctgagagtcgaggacacggctgtgtattactgtgcgagaggtggggaactgggagtcaactactattacgatatggacgtctggggccaagggaccacggtcaccgtctcctca

SEQ ID NO: 66 - protein, 123 aa, Artificial Sequence
  synthetic
QVQLVESGGGAVQPGTSLRLSCAASGFTFSSFGMHWVRQAPGKGLEWVSVIWYEGSNKYYADSVKGRFTISRDNSRNTLSLQMDSLRVEDTAVYYCARGGELGVNYYYDMDVWGQGTTVTVSS

SEQ ID NO: 67 - DNA, 24 bp, Artificial Sequence
  synthetic
ggattcaccttcagtagttttggc

SEQ ID NO: 68 - protein, 8 aa, Artificial Sequence
  synthetic
GFTFSSFG

SEQ ID NO: 69 - DNA, 24 bp, Artificial Sequence
  synthetic
atatggtatgaggggagtaataaa

SEQ ID NO: 70 - protein, 8 aa, Artificial Sequence
  synthetic
IWYEGSNK

SEQ ID NO: 71 - DNA, 48 bp, Artificial Sequence
  synthetic
gcgagaggtggggaactgggagtcaactactattacgatatggacgtc

SEQ ID NO: 72 - protein, 16 aa, Artificial Sequence
  synthetic
ARGGELGVNYYYDMDV

SEQ ID NO: 73 - DNA, 321 bp, Artificial Sequence
  synthetic
gacatccagatgacccagtctccatcctccctgtctgcatctgtaggagacagagtcaccatcacttgccgggcaagtcaggacattaaaaatgatttaggctggtttcagcagaaggcaggtaaagcccctaagcgcctgttctatgctacatccagtttgcaaagtggggtcccatcacggttcagcggcagtggatctgggacagaattcactctcacaatcagcagcctgcagcctgaagattttgcaacttattactgtctacaggttcatagttaccctcggacgttcggccaagggaccaaggtggaaatcaaa

SEQ ID NO: 74 - protein, 107 aa, Artificial Sequence
  synthetic
DIQMTQSPSSLSASVGDRVTITCRASQDIKNDLGWFQQKAGKAPKRLFYATSSLQSGVPSRFSGSGSGTEFTLTISSLQPEDFATYYCLQVHSYPRTFGQGTKVEIK

SEQ ID NO: 75 - DNA, 18 bp, Artificial Sequence
  synthetic
caggacattaaaaatgat

SEQ ID NO: 76 - protein, 6 aa, Artificial Sequence
  synthetic
QDIKND

SEQ ID NO: 77 - DNA, 9 bp, Artificial Sequence
  synthetic
gctacatcc

SEQ ID NO: 78 - protein, 3 aa, Artificial Sequence
  synthetic
ATS

SEQ ID NO: 79 - DNA, 27 bp, Artificial Sequence
  synthetic
ctacaggttcatagttaccctcggacg

SEQ ID NO: 80 - protein, 9 aa, Artificial Sequence
  synthetic
LQVHSYPRT

SEQ ID NO: 81 - DNA, 369 bp, Artificial Sequence
  synthetic
caggtgcagctggtggagtctgggggaggcgtggtccagcctgggaggtccctgagactctcctgtgaagcgtctggattcaccttcagcaactatggctttcactgggtccgccaggctccaggcaaggggctggattgggtggcagttatatggtatgctggaagtaataagttctatgtagactccgtgcagggccgattcaccatctccagagacaattccaaacaaatattgtttcttcaaatgaacagcctgagagccgaggactcggctgtttattactgtgtgagaggggggatactgggcatagactactactccggtatggacgtctggggccaagggaccacggtcaccgtctcctca

SEQ ID NO: 82 - protein, 123 aa, Artificial Sequence
  synthetic
QVQLVESGGGVVQPGRSLRLSCEASGFTFSNYGFHWVRQAPGKGLDWVAVIWYAGSNKFYVDSVQGRFTISRDNSKQILFLQMNSLRAEDSAVYYCVRGGILGIDYYSGMDVWGQGTTVTVSS

SEQ ID NO: 83 - DNA, 24 bp, Artificial Sequence
  synthetic
ggattcaccttcagcaactatggc

SEQ ID NO: 84 - protein, 8 aa, Artificial Sequence
  synthetic
GFTFSNYG

SEQ ID NO: 85 - DNA, 24 bp, Artificial Sequence
  synthetic
atatggtatgctggaagtaataag

SEQ ID NO: 86 - protein, 8 aa, Artificial Sequence
  synthetic
IWYAGSNK

SEQ ID NO: 87 - DNA, 48 bp, Artificial Sequence
  synthetic
gtgagaggggggatactgggcatagactactactccggtatggacgtc

SEQ ID NO: 88 - protein, 16 aa, Artificial Sequence
  synthetic
VRGGILGIDYYSGMDV

SEQ ID NO: 89 - DNA, 321 bp, Artificial Sequence
  synthetic
gccatccagatgacccagtcaccatcctccctgtctgcatctgtaggagacagagtcaccatcacttgccgggcaagtcaggacattagaaatgatttaggctggtatcagcagagaccagggaaggcccctaagttcctgatctattctacatccagtttacaaagtggggtcccatcaagattcagcggcagtggatctggcacagatttcattctcaccatcagcagcctgcagcctgaggattttgccacttattactgtctacaaagtcacaattatccgtggacgttcggccacgggaccaaggtggaaatcaaa

SEQ ID NO: 90 - protein, 107 aa, Artificial Sequence
  synthetic
AIQMTQSPSSLSASVGDRVTITCRASQDIRNDLGWYQQRPGKAPKFLIYSTSSLQSGVPSRFSGSGSGTDFILTISSLQPEDFATYYCLQSHNYPWTFGHGTKVEIK

SEQ ID NO: 91 - DNA, 18 bp, Artificial Sequence
  synthetic
caggacattagaaatgat

SEQ ID NO: 92 - protein, 6 aa, Artificial Sequence
  synthetic
QDIRND

SEQ ID NO: 93 - DNA, 9 bp, Artificial Sequence
  synthetic
tctacatcc

SEQ ID NO: 94 - protein, 3 aa, Artificial Sequence
  synthetic
STS

SEQ ID NO: 95 - DNA, 27 bp, Artificial Sequence
  synthetic
ctacaaagtcacaattatccgtggacg

SEQ ID NO: 96 - protein, 9 aa, Artificial Sequence
  synthetic
LQSHNYPWT

SEQ ID NO: 97 - DNA, 369 bp, Artificial Sequence
  synthetic
caggtgcagctggtggagtctgggggaggcgtggtccagcctgggaggtccctgagactctcctgtgcagtgtctggattcaccctcagtagttatggcatggactgggtccgccaggctccaggcaaggggctggagtgggtggcagttatatggtatgacggaagtaataaatactattcagactccgtgaagggccgattcaccatctccagagacaattccaagaacacactgtttctgcaaatgaacagcctgagagccgacgacacggctgtgtattattgtgcgagagacggggaactgggactggactactactccggtatggacgtctggggccaagggaccacggtcaccgtctcctca

SEQ ID NO: 98 - protein, 123 aa, Artificial Sequence
  synthetic
QVQLVESGGGVVQPGRSLRLSCAVSGFTLSSYGMDWVRQAPGKGLEWVAVIWYDGSNKYYSDSVKGRFTISRDNSKNTLFLQMNSLRADDTAVYYCARDGELGLDYYSGMDVWGQGTTVTVSS

SEQ ID NO: 99 - DNA, 24 bp, Artificial Sequence
  synthetic
ggattcaccctcagtagttatggc

SEQ ID NO: 100 - protein, 8 aa, Artificial Sequence
  synthetic
GFTLSSYG

SEQ ID NO: 101 - DNA, 24 bp, Artificial Sequence
  synthetic
atatggtatgacggaagtaataaa

SEQ ID NO: 102 - protein, 8 aa, Artificial Sequence
  synthetic
IWYDGSNK

SEQ ID NO: 103 - DNA, 48 bp, Artificial Sequence
  synthetic
gcgagagacggggaactgggactggactactactccggtatggacgtc

SEQ ID NO: 104 - protein, 16 aa, Artificial Sequence
  synthetic
ARDGELGLDYYSGMDV

SEQ ID NO: 105 - DNA, 321 bp, Artificial Sequence
  synthetic
gacatccagatgacccagtctccatcctccctgtctgcatctgtaggagacagagtcaccatcacttgccgggcaagtcaggacattagaaatgatttaggctggtatcagcagaaaccagggaaagcccctaagcgcctgatctatggtgcatccagtttgcaaagtggtgtcccatcaaggttcagcggcagtggatctgggacagagttcactctcacaatcagcagcctgcagcctgaagattttgcaacttattattgtctacagcttaatagttaccctcggacgttcggccaagggaccaaggtggaaatcaaa

SEQ ID NO: 106 - protein, 107 aa, Artificial Sequence
  synthetic
DIQMTQSPSSLSASVGDRVTITCRASQDIRNDLGWYQQKPGKAPKRLIYGASSLQSGVPSRFSGSGSGTEFTLTISSLQPEDFATYYCLQLNSYPRTFGQGTKVEIK

SEQ ID NO: 107 - DNA, 18 bp, Artificial Sequence
  synthetic
caggacattagaaatgat

SEQ ID NO: 108 - protein, 6 aa, Artificial Sequence
  synthetic
QDIRND

SEQ ID NO: 109 - DNA, 9 bp, Artificial Sequence
  synthetic
ggtgcatcc

SEQ ID NO: 110 - protein, 3 aa, Artificial Sequence
  synthetic
GAS

SEQ ID NO: 111 - DNA, 27 bp, Artificial Sequence
  synthetic
ctacagcttaatagttaccctcggacg

SEQ ID NO: 112 - protein, 9 aa, Artificial Sequence
  synthetic
LQLNSYPRT

SEQ ID NO: 113 - DNA, 354 bp, Artificial Sequence
  synthetic
caggtgcagctggtggagtctgggggaggcgtggtccagcctgggaggtccctgagactctcctgtgcagcctctggattcaccttcagtagctttggcatgcactgggtccgccaggctccaggcaaggggctggagtgggtggcagtgatatcatatgatggaagaaatagatactatgcagactccgtgaagggccgattcaccatctccagagacaattccaagaacacgctgtatctgcaaatgaacagtctgagcgctgaggacacggctatgttttactgtgcgaaagatggctttggcaactcttttgactactggggccagggaaccctggtcaccgtctcctca

SEQ ID NO: 114 - protein, 118 aa, Artificial Sequence
  synthetic
QVQLVESGGGVVQPGRSLRLSCAASGFTFSSFGMHWVRQAPGKGLEWVAVISYDGRNRYYADSVKGRFTISRDNSKNTLYLQMNSLSAEDTAMFYCAKDGFGNSFDYWGQGTLVTVSS

SEQ ID NO: 115 - DNA, 24 bp, Artificial Sequence
  synthetic
ggattcaccttcagtagctttggc

SEQ ID NO: 116 - protein, 8 aa, Artificial Sequence
  synthetic
GFTFSSFG

SEQ ID NO: 117 - DNA, 24 bp, Artificial Sequence
  synthetic
atatcatatgatggaagaaataga

SEQ ID NO: 118 - protein, 8 aa, Artificial Sequence
  synthetic
ISYDGRNR

SEQ ID NO: 119 - DNA, 33 bp, Artificial Sequence
  synthetic
gcgaaagatggctttggcaactcttttgactac

SEQ ID NO: 120 - protein, 11 aa, Artificial Sequence
  synthetic
AKDGFGNSFDY

SEQ ID NO: 121 - DNA, 336 bp, Artificial Sequence
  synthetic
gatgttgtgatgactcagtctccactctccctgcccgtcacccttggacagccggcctccatctcctgcaggtctagtcaaagcctcctatacagtgatggaaatacctacttgacttggtttcagcagaggccaggccaatctccaaggcgcctaatttataaggtttctaaccgggactctggggtcccagacagattcagcggcagtgggtcaggcactgatttcacactgacaatcagcagggtggaggctgaggatgttgggatttattactgcatgcaaggcacacactggccgtggacgtttggccaagggaccaaggtggaaatcaaa

SEQ ID NO: 122 - protein, 112 aa, Artificial Sequence
  synthetic
DVVMTQSPLSLPVTLGQPASISCRSSQSLLYSDGNTYLTWFQQRPGQSPRRLIYKVSNRDSGVPDRFSGSGSGTDFTLTISRVEAEDVGIYYCMQGTHWPWTFGQGTKVEIK

SEQ ID NO: 123 - DNA, 33 bp, Artificial Sequence
  synthetic
caaagcctcctatacagtgatggaaatacctac

SEQ ID NO: 124 - protein, 11 aa, Artificial Sequence
  synthetic
QSLLYSDGNTY

SEQ ID NO: 125 - DNA, 9 bp, Artificial Sequence
  synthetic
aaggtttct

SEQ ID NO: 126 - protein, 3 aa, Artificial Sequence
  synthetic
KVS

SEQ ID NO: 127 - DNA, 27 bp, Artificial Sequence
  synthetic
atgcaaggcacacactggccgtggacg

SEQ ID NO: 128 - protein, 9 aa, Artificial Sequence
  synthetic
MQGTHWPWT

SEQ ID NO: 129 - DNA, 369 bp, Artificial Sequence
  synthetic
caggtgcagctggtggagtctgggggaggcgtggtccagcctgggaggtccctgagactctcctgtgaagcgtctggattcaccttcagtagctatggcatgcactgggtccgccaggctccaggcaaggggctggagtgggtggcagttatatggtacagtgaaagtaataaatactatacagactccatgaagggccgactcaccatctccagagacaattccaagaacacgctgtatttgcaaatgaacagcctgagagccgaggacacggctgtgtattattgtgcgagaggggggctcctggggaagtactactactacggtatggacgtctggggccaagggaccacggtcaccgtctcctca

SEQ ID NO: 130 - protein, 123 aa, Artificial Sequence
  synthetic
QVQLVESGGGVVQPGRSLRLSCEASGFTFSSYGMHWVRQAPGKGLEWVAVIWYSESNKYYTDSMKGRLTISRDNSKNTLYLQMNSLRAEDTAVYYCARGGLLGKYYYYGMDVWGQGTTVTVSS

SEQ ID NO: 131 - DNA, 24 bp, Artificial Sequence
  synthetic
ggattcaccttcagtagctatggc

SEQ ID NO: 132 - protein, 8 aa, Artificial Sequence
  synthetic
GFTFSSYG

SEQ ID NO: 133 - DNA, 24 bp, Artificial Sequence
  synthetic
atatggtacagtgaaagtaataaa

SEQ ID NO: 134 - protein, 8 aa, Artificial Sequence
  synthetic
IWYSESNK

SEQ ID NO: 135 - DNA, 48 bp, Artificial Sequence
  synthetic
gcgagaggggggctcctggggaagtactactactacggtatggacgtc

SEQ ID NO: 136 - protein, 16 aa, Artificial Sequence
  synthetic
ARGGLLGKYYYYGMDV

SEQ ID NO: 137 - DNA, 321 bp, Artificial Sequence
  synthetic
gacatccagatgacccagtctccatcctccctgtctgcatctgtaggagacagagtcattatcacttgccgggcaagtcaggacattagaaatgatttaggctggtatcagcagaaaccagggaaagcccctaagcgcctgatctatgctgcatccagtttgcaaagtggggtcccatcaaggttcagcggcagtggatctgggacagaattcactctcacaatcagcagcctgcagcctgaagattttgcaactttttactgtctacagcttaatagttacccgtacacttttggccaggggaccaagctggagatcaaa

SEQ ID NO: 138 - protein, 107 aa, Artificial Sequence
  synthetic
DIQMTQSPSSLSASVGDRVIITCRASQDIRNDLGWYQQKPGKAPKRLIYAASSLQSGVPSRFSGSGSGTEFTLTISSLQPEDFATFYCLQLNSYPYTFGQGTKLEIK

SEQ ID NO: 139 - DNA, 18 bp, Artificial Sequence
  synthetic
caggacattagaaatgat

SEQ ID NO: 140 - protein, 6 aa, Artificial Sequence
  synthetic
QDIRND

SEQ ID NO: 141 - DNA, 9 bp, Artificial Sequence
  synthetic
gctgcatcc

SEQ ID NO: 142 - protein, 3 aa, Artificial Sequence
  synthetic
AAS

SEQ ID NO: 143 - DNA, 27 bp, Artificial Sequence
  synthetic
ctacagcttaatagttacccgtacact

SEQ ID NO: 144 - protein, 9 aa, Artificial Sequence
  synthetic
LQLNSYPYT

SEQ ID NO: 145 - DNA, 369 bp, Artificial Sequence
  synthetic
caggtgcagctggtggagtctgggggaggcgtggcccagcctgggaggtccctgagcctctcctgtgcagcgtctggattcaccttcagtgactatggcatgcactgggtccgccaggctccaggcaaggggctggagtgggtggcggttatttggtatgctggaagtaataaatattatgcagactctgtgaaggaccgatttaccatctccagagacaattccaagaacacgctgtatctgcagatgcgcagcctgagagtcgaggacacggctgtatattactgtgcgagagggggggaattgcgtcttgactactactccggtttggacgtctggggccaagggaccacggtcaccgtctcctca

SEQ ID NO: 146 - protein, 123 aa, Artificial Sequence
  synthetic
QVQLVESGGGVAQPGRSLSLSCAASGFTFSDYGMHWVRQAPGKGLEWVAVIWYAGSNKYYADSVKDRFTISRDNSKNTLYLQMRSLRVEDTAVYYCARGGELRLDYYSGLDVWGQGTTVTVSS

SEQ ID NO: 147 - DNA, 24 bp, Artificial Sequence
  synthetic
ggattcaccttcagtgactatggc

SEQ ID NO: 148 - protein, 8 aa, Artificial Sequence
  synthetic
GFTFSDYG

SEQ ID NO: 149 - DNA, 24 bp, Artificial Sequence
  synthetic
atttggtatgctggaagtaataaa

SEQ ID NO: 150 - protein, 8 aa, Artificial Sequence
  synthetic
IWYAGSNK

SEQ ID NO: 151 - DNA, 48 bp, Artificial Sequence
  synthetic
gcgagagggggggaattgcgtcttgactactactccggtttggacgtc

SEQ ID NO: 152 - protein, 16 aa, Artificial Sequence
  synthetic
ARGGELRLDYYSGLDV

SEQ ID NO: 153 - DNA, 321 bp, Artificial Sequence
  synthetic
gacatccagatgacccagtctccatcctccctgtctgcatctgtaggagacagagtcaccgtcacttgccgggcaagtcagggcattagaagtgatttaggctggtatcagcagaaaccaggaaaagcccctaagcgcctgatctatgctgcatccagtttccaaagtggggtcccatcaaggttcagcggcagtggatctgggacagaattcactctcacaatcagcagcctgcaccctgaagattttgctacttattactgtctacagtctaataattacccgtggacgttcggccaagggaccaaggtggaaatcaaa

SEQ ID NO: 154 - protein, 107 aa, Artificial Sequence
  synthetic
DIQMTQSPSSLSASVGDRVTVTCRASQGIRSDLGWYQQKPGKAPKRLIYAASSFQSGVPSRFSGSGSGTEFTLTISSLHPEDFATYYCLQSNNYPWTFGQGTKVEIK

SEQ ID NO: 155 - DNA, 18 bp, Artificial Sequence
  synthetic
cagggcattagaagtgat

SEQ ID NO: 156 - protein, 6 aa, Artificial Sequence
  synthetic
QGIRSD

SEQ ID NO: 157 - DNA, 9 bp, Artificial Sequence
  synthetic
gctgcatcc

SEQ ID NO: 158 - protein, 3 aa, Artificial Sequence
  synthetic
AAS

SEQ ID NO: 159 - DNA, 27 bp, Artificial Sequence
  synthetic
ctacagtctaataattacccgtggacg

SEQ ID NO: 160 - protein, 9 aa, Artificial Sequence
  synthetic
LQSNNYPWT

SEQ ID NO: 161 - DNA, 372 bp, Artificial Sequence
  synthetic
caggtgcagctggtggagtctgggggaggcgtggtccagccgggggggtcccttagactctcctgtgcagtgtctggattcaccttcagtgactatggcatgcactgggtccgccaggttccaggcgcggggctggagtgggtggcagttatttactatgaaggaagtaacaaatactatgcagactccgtgaagggccgattcaccatctccagagacaattccaagaacacgctgtatctgcaaatgaacagcctgagagtcgaggacacgtctatgtatttctgtgcgagaggcccccttctcggcgggaacttctactcttaccttatggacgtctggggccaggggaccacggtcaccgtctcctca

SEQ ID NO: 162 - protein, 124 aa, Artificial Sequence
  synthetic
QVQLVESGGGVVQPGGSLRLSCAVSGFTFSDYGMHWVRQVPGAGLEWVAVIYYEGSNKYYADSVKGRFTISRDNSKNTLYLQMNSLRVEDTSMYFCARGPLLGGNFYSYLMDVWGQGTTVTVSS

SEQ ID NO: 163 - DNA, 24 bp, Artificial Sequence
  synthetic
ggattcaccttcagtgactatggc

SEQ ID NO: 164 - protein, 8 aa, Artificial Sequence
  synthetic
GFTFSDYG

SEQ ID NO: 165 - DNA, 24 bp, Artificial Sequence
  synthetic
atttactatgaaggaagtaacaaa

SEQ ID NO: 166 - protein, 8 aa, Artificial Sequence
  synthetic
IYYEGSNK

SEQ ID NO: 167 - DNA, 51 bp, Artificial Sequence
  synthetic
gcgagaggcccccttctcggcgggaacttctactcttaccttatggacgtc

SEQ ID NO: 168 - protein, 17 aa, Artificial Sequence
  synthetic
ARGPLLGGNFYSYLMDV

SEQ ID NO: 169 - DNA, 321 bp, Artificial Sequence
  synthetic
gccatccagatgacccagtctccatcctccctgtctgcatctgtaggagacagagtcaccatcacttgccgggcaagtcagggcattagaaatggtttaggctggtatcagcagaaaccagggaaagcccctaaactcctgatctatactgcatccagtttacaaagtggagtcccatcaagattcagcggcagtggatctggcacagacttcactctcaccatcagcagcctgcagcctgaagattttgcaacttattactgtctacaagattacaattaccctttcagtttcggccctgggaccaaagtggatatcaaa

SEQ ID NO: 170 - protein, 107 aa, Artificial Sequence
  synthetic
AIQMTQSPSSLSASVGDRVTITCRASQGIRNGLGWYQQKPGKAPKLLIYTASSLQSGVPSRFSGSGSGTDFTLTISSLQPEDFATYYCLQDYNYPFSFGPGTKVDIK

SEQ ID NO: 171 - DNA, 18 bp, Artificial Sequence
  synthetic
cagggcattagaaatggt

SEQ ID NO: 172 - protein, 6 aa, Artificial Sequence
  synthetic
QGIRNG

SEQ ID NO: 173 - DNA, 9 bp, Artificial Sequence
  synthetic
actgcatcc

SEQ ID NO: 174 - protein, 3 aa, Artificial Sequence
  synthetic
TAS

SEQ ID NO: 175 - DNA, 27 bp, Artificial Sequence
  synthetic
ctacaagattacaattaccctttcagt

SEQ ID NO: 176 - protein, 9 aa, Artificial Sequence
  synthetic
LQDYNYPFS

SEQ ID NO: 177 - DNA, 372 bp, Artificial Sequence
  synthetic
caggtgcagctggtggagtctgggggaggcgtggtccagcctgggaggtccctgagactctcctgtgcagcgtctggatttaccgtcagaaactatggcatgcactgggtccgccaggctccaggcaaggggctggagtgggtggcagttatatggtatgatggaagtaataaatactatgcagactccgtgaagggccgattcaccatctccagagacaattccaagaacacgctgtttctgcaaatgaacagcctgagagccgaggacacggctgtgtattactgtgcgagagggggagagctggtacgtggggactactactacggtatggacgtctggggccaagggaccacggtcaccgtctcctca

SEQ ID NO: 178 - protein, 124 aa, Artificial Sequence
  synthetic
QVQLVESGGGVVQPGRSLRLSCAASGFTVRNYGMHWVRQAPGKGLEWVAVIWYDGSNKYYADSVKGRFTISRDNSKNTLFLQMNSLRAEDTAVYYCARGGELVRGDYYYGMDVWGQGTTVTVSS

SEQ ID NO: 179 - DNA, 24 bp, Artificial Sequence
  synthetic
ggatttaccgtcagaaactatggc

SEQ ID NO: 180 - protein, 8 aa, Artificial Sequence
  synthetic
GFTVRNYG

SEQ ID NO: 181 - DNA, 24 bp, Artificial Sequence
  synthetic
atatggtatgatggaagtaataaa

SEQ ID NO: 182 - protein, 8 aa, Artificial Sequence
  synthetic
IWYDGSNK

SEQ ID NO: 183 - DNA, 51 bp, Artificial Sequence
  synthetic
gcgagagggggagagctggtacgtggggactactactacggtatggacgtc

SEQ ID NO: 184 - protein, 17 aa, Artificial Sequence
  synthetic
ARGGELVRGDYYYGMDV

SEQ ID NO: 185 - DNA, 321 bp, Artificial Sequence
  synthetic
gacatccagatgacccagtctccatcctccctgtctgcatctgtaggagacagagtcaccatcacttgccgggcaagtcagggcattagaaatgatttaggctggtatcagcagaaaccagggaaagcccctaagcgcctgatctatggtgcatccagtttgcaaagtggggtcccatcaaggttcagcggcagtggatctgggacagaattcactctcacaatcagcagcctgcagcctgaagattttgcaacttattactgtctacagcataatagttacccgtacacttttggccaggggaccaagctggagatcaaa

SEQ ID NO: 186 - protein, 107 aa, Artificial Sequence
  synthetic
DIQMTQSPSSLSASVGDRVTITCRASQGIRNDLGWYQQKPGKAPKRLIYGASSLQSGVPSRFSGSGSGTEFTLTISSLQPEDFATYYCLQHNSYPYTFGQGTKLEIK

SEQ ID NO: 187 - DNA, 18 bp, Artificial Sequence
  synthetic
cagggcattagaaatgat

SEQ ID NO: 188 - protein, 6 aa, Artificial Sequence
  synthetic
QGIRND

SEQ ID NO: 189 - DNA, 9 bp, Artificial Sequence
  synthetic
ggtgcatcc

SEQ ID NO: 190 - protein, 3 aa, Artificial Sequence
  synthetic
GAS

SEQ ID NO: 191 - DNA, 27 bp, Artificial Sequence
  synthetic
ctacagcataatagttacccgtacact

SEQ ID NO: 192 - protein, 9 aa, Artificial Sequence
  synthetic
LQHNSYPYT

SEQ ID NO: 193 - DNA, 351 bp, Artificial Sequence
  synthetic
caggtgcagctggtggagtctgggggcggcgtggtccagcctgggaggtccctgagactctcctgtgcagcctctggaactatcttcagtacccatggcatgcactgggtccgccaggctccaggcaaggggctggagtgggtggcagttatatcatatgatggaaataagaagtactatgcaggctccgtgaagggccgattcaccatctccagagacaattccaagaacacgctgtatctgcaaatgaacgacgttagatctgaggacacggctgtttatcactgtacgacagatattactggaatcacggactactggggccagggaaccctggtcaccgtctcctca

SEQ ID NO: 194 - protein, 117 aa, Artificial Sequence
  synthetic
QVQLVESGGGVVQPGRSLRLSCAASGTIFSTHGMHWVRQAPGKGLEWVAVISYDGNKKYYAGSVKGRFTISRDNSKNTLYLQMNDVRSEDTAVYHCTTDITGITDYWGQGTLVTVSS

SEQ ID NO: 195 - DNA, 24 bp, Artificial Sequence
  synthetic
ggaactatcttcagtacccatggc

SEQ ID NO: 196 - protein, 8 aa, Artificial Sequence
  synthetic
GTIFSTHG

SEQ ID NO: 197 - DNA, 24 bp, Artificial Sequence
  synthetic
atatcatatgatggaaataagaag

SEQ ID NO: 198 - protein, 8 aa, Artificial Sequence
  synthetic
ISYDGNKK

SEQ ID NO: 199 - DNA, 30 bp, Artificial Sequence
  synthetic
acgacagatattactggaatcacggactac

SEQ ID NO: 200 - protein, 10 aa, Artificial Sequence
  synthetic
TTDITGITDY

SEQ ID NO: 201 - DNA, 318 bp, Artificial Sequence
  synthetic
gacatccagatgacccagtctccatcctccctgtctgcatctgtaggagacagagtcaccatcacttgccgggcaagtcagggcattggaaatgatttaggctggtatcagcagaaactagggaaggcccctaagcgcctgatctatgctgcatccagtttggagagtggggtcccatcaaggttcagcggcagtggatccgggacagaattcattctcacaatcagcagcctgcaggctgaagattttgcaacttactactgtctacagcataatggtttcccgacgttcggccaagggaccaaggtggaaatcaaa

SEQ ID NO: 202 - protein, 106 aa, Artificial Sequence
  synthetic
DIQMTQSPSSLSASVGDRVTITCRASQGIGNDLGWYQQKLGKAPKRLIYAASSLESGVPSRFSGSGSGTEFILTISSLQAEDFATYYCLQHNGFPTFGQGTKVEIK

SEQ ID NO: 203 - DNA, 18 bp, Artificial Sequence
  synthetic
cagggcattggaaatgat

SEQ ID NO: 204 - protein, 6 aa, Artificial Sequence
  synthetic
QGIGND

SEQ ID NO: 205 - DNA, 9 bp, Artificial Sequence
  synthetic
gctgcatcc

SEQ ID NO: 206 - protein, 3 aa, Artificial Sequence
  synthetic
AAS

SEQ ID NO: 207 - DNA, 24 bp, Artificial Sequence
  synthetic
ctacagcataatggtttcccgacg

SEQ ID NO: 208 - protein, 8 aa, Artificial Sequence
  synthetic
LQHNGFPT

SEQ ID NO: 209 - DNA, 363 bp, Artificial Sequence
  synthetic
caggtgcagctggtggagtctgggggaggcgtggtccagcctgggaggtccctgagactctcctgtgcagcgtctggattcaccttcagtaactatggcattcactgggtccgccagcctccaggccagggcctggagtgggtggcagttatatggtatgctggaagtaataagttttatgcagattccgtgaagggccgattcaccatctccagagacaattccaagaactcggcgtatctgcaaatgaacagcctgagagccgaggatacggctgtgtattactgtgcgagagcccccctgggttattactactacggtatggacgtctggggccaagggaccacggtcaccgtctcctca

SEQ ID NO: 210 - protein, 121 aa, Artificial Sequence
  synthetic
QVQLVESGGGVVQPGRSLRLSCAASGFTFSNYGIHWVRQPPGQGLEWVAVIWYAGSNKFYADSVKGRFTISRDNSKNSAYLQMNSLRAEDTAVYYCARAPLGYYYYGMDVWGQGTTVTVSS

SEQ ID NO: 211 - DNA, 24 bp, Artificial Sequence
  synthetic
ggattcaccttcagtaactatggc

SEQ ID NO: 212 - protein, 8 aa, Artificial Sequence
  synthetic
GFTFSNYG

SEQ ID NO: 213 - DNA, 24 bp, Artificial Sequence
  synthetic
atatggtatgctggaagtaataag

SEQ ID NO: 214 - protein, 8 aa, Artificial Sequence
  synthetic
IWYAGSNK

SEQ ID NO: 215 - DNA, 42 bp, Artificial Sequence
  synthetic
gcgagagcccccctgggttattactactacggtatggacgtc

SEQ ID NO: 216 - protein, 14 aa, Artificial Sequence
  synthetic
ARAPLGYYYYGMDV

SEQ ID NO: 217 - DNA, 321 bp, Artificial Sequence
  synthetic
gacatccagatgacccagtctccatcctccctgtctgcatctgtaggagacagagtcaccatcacttgccgggcaagtcagggcattagaaatgatttaggctggtatcagcagaaaccagggaaagcccctaagcgcctgatctatgatgcatccagtttggaaagtggggtcccatcaaggttcagcggcagtggatctgggacagaattcactctcacaatcagcagcctgcagcctgaagattttgcaacttattactgtctacagcataatagttacccgtggacgttcggccaagggaccaaggtggaaatcaaa

SEQ ID NO: 218 - protein, 107 aa, Artificial Sequence
  synthetic
DIQMTQSPSSLSASVGDRVTITCRASQGIRNDLGWYQQKPGKAPKRLIYDASSLESGVPSRFSGSGSGTEFTLTISSLQPEDFATYYCLQHNSYPWTFGQGTKVEIK

SEQ ID NO: 219 - DNA, 18 bp, Artificial Sequence
  synthetic
cagggcattagaaatgat

SEQ ID NO: 220 - protein, 6 aa, Artificial Sequence
  synthetic
QGIRND

SEQ ID NO: 221 - DNA, 9 bp, Artificial Sequence
  synthetic
gatgcatcc

SEQ ID NO: 222 - protein, 3 aa, Artificial Sequence
  synthetic
DAS

SEQ ID NO: 223 - DNA, 27 bp, Artificial Sequence
  synthetic
ctacagcataatagttacccgtggacg

SEQ ID NO: 224 - protein, 9 aa, Artificial Sequence
  synthetic
LQHNSYPWT

SEQ ID NO: 225 - DNA, 375 bp, Artificial Sequence
  synthetic
caggtgcagctggtggagtctgggggaggcgtggtccagcctgggaggtccctgagactctcctgtgcagcgtctggactcaccgtcagtagttatgtcatgcactgggtccgccaggctccaggcaaggggctggagtgggtggcaattatatggtatgatggaagtaataaatactatggagactccgtgaagggccgattcaccatctccagagacaattccaagaaaacgctgtatctgcaaatgaacagcctgagagccgaggacacggctgtgtattactgtgcgagaggccgccccctgtctagtagttcgtccgattattacggtttggacgtctggggccaagggaccacggtcaccgtctcctca

SEQ ID NO: 226 - protein, 125 aa, Artificial Sequence
  synthetic
QVQLVESGGGVVQPGRSLRLSCAASGLTVSSYVMHWVRQAPGKGLEWVAIIWYDGSNKYYGDSVKGRFTISRDNSKKTLYLQMNSLRAEDTAVYYCARGRPLSSSSSDYYGLDVWGQGTTVTVSS

SEQ ID NO: 227 - DNA, 24 bp, Artificial Sequence
  synthetic
ggactcaccgtcagtagttatgtc

SEQ ID NO: 228 - protein, 8 aa, Artificial Sequence
  synthetic
GLTVSSYV

SEQ ID NO: 229 - DNA, 24 bp, Artificial Sequence
  synthetic
atatggtatgatggaagtaataaa

SEQ ID NO: 230 - protein, 8 aa, Artificial Sequence
  synthetic
IWYDGSNK

SEQ ID NO: 231 - DNA, 54 bp, Artificial Sequence
  synthetic
gcgagaggccgccccctgtctagtagttcgtccgattattacggtttggacgtc

SEQ ID NO: 232 - protein, 18 aa, Artificial Sequence
  synthetic
ARGRPLSSSSSDYYGLDV

SEQ ID NO: 233 - DNA, 321 bp, Artificial Sequence
  synthetic
gccatccagatgacccagtctccatcctccctgtctgcatctgtaggagacagagtcaccatcatttgccgggcaagtcagggcattagaaatgatttaggctggtatcagcagaaaccagggaaagcccctaacctcctgatctatgctgcatccagtttacaaagtggggtcccatcaaggttcagcggcagtggatctggcacagatttcactctcaccatcagcagcctgcagcctgaagattttgcaacttattactgtctacaagattacaattatccgtggacgttcggccaagggaccaaggtggaaatcaaa

SEQ ID NO: 234 - protein, 107 aa, Artificial Sequence
  synthetic
AIQMTQSPSSLSASVGDRVTIICRASQGIRNDLGWYQQKPGKAPNLLIYAASSLQSGVPSRFSGSGSGTDFTLTISSLQPEDFATYYCLQDYNYPWTFGQGTKVEIK

SEQ ID NO: 235 - DNA, 18 bp, Artificial Sequence
  synthetic
cagggcattagaaatgat

SEQ ID NO: 236 - protein, 6 aa, Artificial Sequence
  synthetic
QGIRND

SEQ ID NO: 237 - DNA, 9 bp, Artificial Sequence
  synthetic
gctgcatcc

SEQ ID NO: 238 - protein, 3 aa, Artificial Sequence
  synthetic
AAS

SEQ ID NO: 239 - DNA, 27 bp, Artificial Sequence
  synthetic
ctacaagattacaattatccgtggacg

SEQ ID NO: 240 - protein, 9 aa, Artificial Sequence
  synthetic
LQDYNYPWT

SEQ ID NO: 241 - DNA, 360 bp, Artificial Sequence
  synthetic
gaggtgcagctggtggagtctgggggaggcctggtacagcctggagggtccctgagactctcctgtgcagcctctggattcaccttcagtaattatgaaatgtattgggtccgccaggctccagggaaggggctggaatgggtttcatacattagtagtagtggtactaccatatactacgcagactctgtgaagggccgattcagtgtctccagagaaaacgccaggagctcactgtatctgcaaatgaacagtctgagagtcgaggactcggctgtttacttctgtgcgaagtataactggaactccttctatggtttggacgtctggggccaagggaccacggtcaccgtctcctca

SEQ ID NO: 242 - protein, 120 aa, Artificial Sequence
  synthetic
EVQLVESGGGLVQPGGSLRLSCAASGFTFSNYEMYWVRQAPGKGLEWVSYISSSGTTIYYADSVKGRFSVSRENARSSLYLQMNSLRVEDSAVYFCAKYNWNSFYGLDVWGQGTTVTVSS

SEQ ID NO: 243 - DNA, 24 bp, Artificial Sequence
  synthetic
ggattcaccttcagtaattatgaa

SEQ ID NO: 244 - protein, 8 aa, Artificial Sequence
  synthetic
GFTFSNYE

SEQ ID NO: 245 - DNA, 24 bp, Artificial Sequence
  synthetic
attagtagtagtggtactaccata

SEQ ID NO: 246 - protein, 8 aa, Artificial Sequence
  synthetic
ISSSGTTI

SEQ ID NO: 247 - DNA, 39 bp, Artificial Sequence
  synthetic
gcgaagtataactggaactccttctatggtttggacgtc

SEQ ID NO: 248 - protein, 13 aa, Artificial Sequence
  synthetic
AKYNWNSFYGLDV

SEQ ID NO: 249 - DNA, 321 bp, Artificial Sequence
  synthetic
gccatccagatgacccagtctccatcctccctgtctgcatctgtaggagacagagtcaccatcacttgccgggcaagtcaggacattagaaatgatttaggctggtatcagcagaaaccagggaaagcccctaagctcctgatctctgctgcatccagtttacagggtggggtcccatcaaggttcagcggcagtggatctggcacagatttcactctcaccattagcagcctgcagcctgcagattttgcaacttattactgtctacaagagtacaattatgcactcactttcggcggagggaccaaggtggagatcaaa

SEQ ID NO: 250 - protein, 107 aa, Artificial Sequence
  synthetic
AIQMTQSPSSLSASVGDRVTITCRASQDIRNDLGWYQQKPGKAPKLLISAASSLQGGVPSRFSGSGSGTDFTLTISSLQPADFATYYCLQEYNYALTFGGGTKVEIK

SEQ ID NO: 251 - DNA, 18 bp, Artificial Sequence
  synthetic
caggacattagaaatgat

SEQ ID NO: 252 - protein, 6 aa, Artificial Sequence
  synthetic
QDIRND

SEQ ID NO: 253 - DNA, 9 bp, Artificial Sequence
  synthetic
gctgcatcc

SEQ ID NO: 254 - protein, 3 aa, Artificial Sequence
  synthetic
AAS

SEQ ID NO: 255 - DNA, 27 bp, Artificial Sequence
  synthetic
ctacaagagtacaattatgcactcact

SEQ ID NO: 256 - protein, 9 aa, Artificial Sequence
  synthetic
LQEYNYALT

SEQ ID NO: 257 - DNA, 369 bp, Artificial Sequence
  synthetic
gaggtgcagctggtggagtctgggggaggtttggtccagcctggagggtccctgagactctcctgtgcagcctctggattcaccttcagggtttatgaaatgaactgggtccgccaggctccagggaaggggctggagtggatttcatacattggcagtagtggttttaccatatactacgcagactctgtgaagggccgattcaccatctccagagacaacgccaagaactcactgtttctgcagctgaacagcctgagagccgaggacacggctgtttattactgtgcgagagggtggaacgacggagttcctaactatttgggtatggacgtctggggccaaggcaccacggtcaccgtctcctca

SEQ ID NO: 258 - protein, 123 aa, Artificial Sequence
  synthetic
EVQLVESGGGLVQPGGSLRLSCAASGFTFRVYEMNWVRQAPGKGLEWISYIGSSGFTIYYADSVKGRFTISRDNAKNSLFLQLNSLRAEDTAVYYCARGWNDGVPNYLGMDVWGQGTTVTVSS

SEQ ID NO: 259 - DNA, 24 bp, Artificial Sequence
  synthetic
ggattcaccttcagggtttatgaa

SEQ ID NO: 260 - protein, 8 aa, Artificial Sequence
  synthetic
GFTFRVYE

SEQ ID NO: 261 - DNA, 24 bp, Artificial Sequence
  synthetic
attggcagtagtggttttaccata

SEQ ID NO: 262 - protein, 8 aa, Artificial Sequence
  synthetic
IGSSGFTI

SEQ ID NO: 263 - DNA, 48 bp, Artificial Sequence
  synthetic
gcgagagggtggaacgacggagttcctaactatttgggtatggacgtc

SEQ ID NO: 264 - protein, 16 aa, Artificial Sequence
  synthetic
ARGWNDGVPNYLGMDV

SEQ ID NO: 265 - DNA, 321 bp, Artificial Sequence
  synthetic
gacatccagatgacccagtctccatcctccctgtctgcatctgtaggagacagagtcaccatcacttgccaggcgagtcaggacattaacaaatatttaaattggtatcagcagaaaccaggaaaagcccctaaactcctgatctacgatgcatccaatttggaaacaggggtcccatcaaggttcagtggaagtggatctgggacagattttactttcaccatcagcagcctgcagcctgaagatattgcaagatatcactgtcaacagtatgataaaatcccgctcactttcggcggagggaccaaggtggagatcaaa

SEQ ID NO: 266 - protein, 107 aa, Artificial Sequence
  synthetic
DIQMTQSPSSLSASVGDRVTITCQASQDINKYLNWYQQKPGKAPKLLIYDASNLETGVPSRFSGSGSGTDFTFTISSLQPEDIARYHCQQYDKIPLTFGGGTKVEIK

SEQ ID NO: 267 - DNA, 18 bp, Artificial Sequence
  synthetic
caggacattaacaaatat

SEQ ID NO: 268 - protein, 6 aa, Artificial Sequence
  synthetic
QDINKY

SEQ ID NO: 269 - DNA, 9 bp, Artificial Sequence
  synthetic
gatgcatcc

SEQ ID NO: 270 - protein, 3 aa, Artificial Sequence
  synthetic
DAS

SEQ ID NO: 271 - DNA, 27 bp, Artificial Sequence
  synthetic
caacagtatgataaaatcccgctcact

SEQ ID NO: 272 - protein, 9 aa, Artificial Sequence
  synthetic
QQYDKIPLT

SEQ ID NO: 273 - DNA, 369 bp, Artificial Sequence
  synthetic
caggtgcagctggtggagtctgggggaggcgtggtccagcctgggaggtccctgagactctcctgtgcagcgtctggattcaccttcagcagctatggcatgcactgggtccgccaggctccaggcaaggggctggagtgggtggcagttatctggtatgttggaagtaataaatactatggagagtccgtgaagggccgattcaccatctccagagacaattccaagaacacgctgtatttgcaaatgaacagcctgagagacgaggacacggctatatattactgtgcgagagggggtcaactgggctccttctactattacggtatggacgtctggggccaagggaccacggtcaccgtctcctca

SEQ ID NO: 274 - protein, 123 aa, Artificial Sequence
  synthetic
QVQLVESGGGVVQPGRSLRLSCAASGFTFSSYGMHWVRQAPGKGLEWVAVIWYVGSNKYYGESVKGRFTISRDNSKNTLYLQMNSLRDEDTAIYYCARGGQLGSFYYYGMDVWGQGTTVTVSS

SEQ ID NO: 275 - DNA, 24 bp, Artificial Sequence
  synthetic
ggattcaccttcagcagctatggc

SEQ ID NO: 276 - protein, 8 aa, Artificial Sequence
  synthetic
GFTFSSYG

SEQ ID NO: 277 - DNA, 24 bp, Artificial Sequence
  synthetic
atctggtatgttggaagtaataaa

SEQ ID NO: 278 - protein, 8 aa, Artificial Sequence
  synthetic
IWYVGSNK

SEQ ID NO: 279 - DNA, 48 bp, Artificial Sequence
  synthetic
gcgagagggggtcaactgggctccttctactattacggtatggacgtc

SEQ ID NO: 280 - protein, 16 aa, Artificial Sequence
  synthetic
ARGGQLGSFYYYGMDV

SEQ ID NO: 281 - DNA, 321 bp, Artificial Sequence
  synthetic
gacatccagatgacccagtctccatcctccctgtctgcatctgtaggagacagagtcaccatcacttgccgggcaagtcagggcattagaaatgatttaggctggtatcagcagaaaccagggaaagcccctaagcgcctgatctatgatgtatccagtttacaaagtggggtcccatcaaggttcagcggcagtggatctgggacagaattcactctcacaatcagcagcctgcagcctgaagatcttgcaacttattactgtctacagcataatagttacccgtggacgttcggccaagggaccaaggtggaaatcaaa

SEQ ID NO: 282 - protein, 107 aa, Artificial Sequence
  synthetic
DIQMTQSPSSLSASVGDRVTITCRASQGIRNDLGWYQQKPGKAPKRLIYDVSSLQSGVPSRFSGSGSGTEFTLTISSLQPEDLATYYCLQHNSYPWTFGQGTKVEIK

SEQ ID NO: 283 - DNA, 18 bp, Artificial Sequence
  synthetic
cagggcattagaaatgat

SEQ ID NO: 284 - protein, 6 aa, Artificial Sequence
  synthetic
QGIRND

SEQ ID NO: 285 - DNA, 9 bp, Artificial Sequence
  synthetic
gatgtatcc

SEQ ID NO: 286 - protein, 3 aa, Artificial Sequence
  synthetic
DVS

SEQ ID NO: 287 - DNA, 27 bp, Artificial Sequence
  synthetic
ctacagcataatagttacccgtggacg

SEQ ID NO: 288 - protein, 9 aa, Artificial Sequence
  synthetic
LQHNSYPWT

SEQ ID NO: 289 - DNA, 360 bp, Artificial Sequence
  synthetic
caggtgcagctggtggagtctgggggaggcgtggtccagcctgggaggtccctgagaatttcctgtgcagcgtcaggattcaccttcaataactatggcttccactgggtccgccaggctccaggcagggggctggagtgggtggcagttatttggtattctggaagtaataaatactatggagactccgtgaagggccgattcaccatctccagagacaattccaaaaatatattgtatctgcaaatgaacagtctgagagccgaggacacggctatatattactgtgcgagatttccgtttagcagcagttggctcttggactactggggccagggaaccctggtcaccgtctcctca

SEQ ID NO: 290 - protein, 120 aa, Artificial Sequence
  synthetic
QVQLVESGGGVVQPGRSLRISCAASGFTFNNYGFHWVRQAPGRGLEWVAVIWYSGSNKYYGDSVKGRFTISRDNSKNILYLQMNSLRAEDTAIYYCARFPFSSSWLLDYWGQGTLVTVSS

SEQ ID NO: 291 - DNA, 24 bp, Artificial Sequence
  synthetic
ggattcaccttcaataactatggc

SEQ ID NO: 292 - protein, 8 aa, Artificial Sequence
  synthetic
GFTFNNYG

SEQ ID NO: 293 - DNA, 24 bp, Artificial Sequence
  synthetic
atttggtattctggaagtaataaa

SEQ ID NO: 294 - protein, 8 aa, Artificial Sequence
  synthetic
IWYSGSNK

SEQ ID NO: 295 - DNA, 39 bp, Artificial Sequence
  synthetic
gcgagatttccgtttagcagcagttggctcttggactac

SEQ ID NO: 296 - protein, 13 aa, Artificial Sequence
  synthetic
ARFPFSSSWLLDY

SEQ ID NO: 297 - DNA, 321 bp, Artificial Sequence
  synthetic
gacatccagttgacccagtctccatccttcctgtctgcatctgtaggagacagagtcaccttcacttgctgggccagtcagggcattagtgattatttagcctggtatcaacaaaaaccagggaaagcccctaaactcctgatctatgctgcatccgctttgcaaagtggggtcccatcaaggttcagcggcagtggatctgggacagaattcactctcacagtcagcagcctacagcctgaagattttgcaacttattactgtcaacagcttaatagttatccattcactttcggccctgggaccaaagtggatatcaaa

SEQ ID NO: 298 - protein, 107 aa, Artificial Sequence
  synthetic
DIQLTQSPSFLSASVGDRVTFTCWASQGISDYLAWYQQKPGKAPKLLIYAASALQSGVPSRFSGSGSGTEFTLTVSSLQPEDFATYYCQQLNSYPFTFGPGTKVDIK

SEQ ID NO: 299 - DNA, 18 bp, Artificial Sequence
  synthetic
cagggcattagtgattat

SEQ ID NO: 300 - protein, 6 aa, Artificial Sequence
  synthetic
QGISDY

SEQ ID NO: 301 - DNA, 9 bp, Artificial Sequence
  synthetic
gctgcatcc

SEQ ID NO: 302 - protein, 3 aa, Artificial Sequence
  synthetic
AAS

SEQ ID NO: 303 - DNA, 27 bp, Artificial Sequence
  synthetic
caacagcttaatagttatccattcact

SEQ ID NO: 304 - protein, 9 aa, Artificial Sequence
  synthetic
QQLNSYPFT

SEQ ID NO: 305 - DNA, 357 bp, Artificial Sequence
  synthetic
cagctgcagctgcaggagtcgggcccaggactggtgaagccttcggagaccctgtccctcacctgcactgtctctggtggctccatcagcagtactaatcactactggggctggatccgccagcccccagggaagggcctggagtggatcggtaatgtctattatattgggaacgcctactacaacccgtccctcaagactggagtcaccttttccgtagacacgtccaagaaccagttctccctgaacctgaggtctgtgaccgccgcagacacggctatgtattactgtgcgagactttctaactggaatttcttggacttgtggggccagggaaccctggtcaccgtctcctca

SEQ ID NO: 306 - protein, 119 aa, Artificial Sequence
  synthetic
QLQLQESGPGLVKPSETLSLTCTVSGGSISSTNHYWGWIRQPPGKGLEWIGNVYYIGNAYYNPSLKTGVTFSVDTSKNQFSLNLRSVTAADTAMYYCARLSNWNFLDLWGQGTLVTVSS

SEQ ID NO: 307 - DNA, 30 bp, Artificial Sequence
  synthetic
ggtggctccatcagcagtactaatcactac

SEQ ID NO: 308 - protein, 10 aa, Artificial Sequence
  synthetic
GGSISSTNHY

SEQ ID NO: 309 - DNA, 21 bp, Artificial Sequence
  synthetic
gtctattatattgggaacgcc

SEQ ID NO: 310 - protein, 7 aa, Artificial Sequence
  synthetic
VYYIGNA

SEQ ID NO: 311 - DNA, 33 bp, Artificial Sequence
  synthetic
gcgagactttctaactggaatttcttggacttg

SEQ ID NO: 312 - protein, 11 aa, Artificial Sequence
  synthetic
ARLSNWNFLDL

SEQ ID NO: 313 - DNA, 318 bp, Artificial Sequence
  synthetic
gaaattgtgatgacgcagtctccagccaccctgtctgtgtctccaggggaaagagccaccctctcctgcagggccagtcagagtattagcagcaacttagcctggtaccagcagaaacctggccaggctcccaggctcctcatctatggtgcatccaccagggccactggtatcccagccaggttcagtggcagtgggtctgggacagagttcactctcaccatcagcagcctgcagtctgaagattttgcagtttattactgtcagcaatttaataactggctctctttcggcggagggaccaaggtggagatcaaa

SEQ ID NO: 314 - protein, 106 aa, Artificial Sequence
  synthetic
EIVMTQSPATLSVSPGERATLSCRASQSISSNLAWYQQKPGQAPRLLIYGASTRATGIPARFSGSGSGTEFTLTISSLQSEDFAVYYCQQFNNWLSFGGGTKVEIK

SEQ ID NO: 315 - DNA, 18 bp, Artificial Sequence
  synthetic
cagagtattagcagcaac

SEQ ID NO: 316 - protein, 6 aa, Artificial Sequence
  synthetic
QSISSN

SEQ ID NO: 317 - DNA, 9 bp, Artificial Sequence
  synthetic
ggtgcatcc

SEQ ID NO: 318 - protein, 3 aa, Artificial Sequence
  synthetic
GAS

SEQ ID NO: 319 - DNA, 24 bp, Artificial Sequence
  synthetic
cagcaatttaataactggctctct

SEQ ID NO: 320 - protein, 8 aa, Artificial Sequence
  synthetic
QQFNNWLS

SEQ ID NO: 321 - DNA, 366 bp, Artificial Sequence
  synthetic
caggtgcagctggtggagtcgggggggggcgtggtccagcctgggaggtccctgagactctcctgtgcagcgtctggattcaccttcagtacctatggcatgcactgggtccgccaggctccaggcaaggggctggagtgggtggcagttatatggtatgttggaagtaataaattctatgcagactccgtgaagggccgattcaccatctccagagacaattccaagaacacgctgtatctgcaaatggacagcctgagagccgaggacacgggtgtgtatcactgtgcgagagacagtatggttcggccctattattacggtatggacgtctggggccaagggaccacggtcaccgtctcctca

SEQ ID NO: 322 - protein, 122 aa, Artificial Sequence
  synthetic
QVQLVESGGGVVQPGRSLRLSCAASGFTFSTYGMHWVRQAPGKGLEWVAVIWYVGSNKFYADSVKGRFTISRDNSKNTLYLQMDSLRAEDTGVYHCARDSMVRPYYYGMDVWGQGTTVTVSS

SEQ ID NO: 323 - DNA, 24 bp, Artificial Sequence
  synthetic
ggattcaccttcagtacctatggc

SEQ ID NO: 324 - protein, 8 aa, Artificial Sequence
  synthetic
GFTFSTYG

SEQ ID NO: 325 - DNA, 24 bp, Artificial Sequence
  synthetic
atatggtatgttggaagtaataaa

SEQ ID NO: 326 - protein, 8 aa, Artificial Sequence
  synthetic
IWYVGSNK

SEQ ID NO: 327 - DNA, 45 bp, Artificial Sequence
  synthetic
gcgagagacagtatggttcggccctattattacggtatggacgtc

SEQ ID NO: 328 - protein, 15 aa, Artificial Sequence
  synthetic
ARDSMVRPYYYGMDV

SEQ ID NO: 329 - DNA, 375 bp, Artificial Sequence
  synthetic
caggtgcagctggtggagtctgggggaggcgtggtccaacctgggaggtccctgagactctcctgttcagcgtctggattcaccctcagtaattttgtcatgcattgggtccgccaggctccaggcaaggggctggagtgggtggcagtcatattatatgatggaagtaataaatattatgcggactccgtgaagggccgattcaccatctccagagacaattccaacaacaggctgtatctgcaaatgaacagcctgagagccgaggacacggctctttattactgtgcgagaggagagtccttgggatcacctatctattattactacggtttggacgtctggggccaagggaccacggtcaccgtctcctca

SEQ ID NO: 330 - protein, 125 aa, Artificial Sequence
  synthetic
QVQLVESGGGVVQPGRSLRLSCSASGFTLSNFVMHWVRQAPGKGLEWVAVILYDGSNKYYADSVKGRFTISRDNSNNRLYLQMNSLRAEDTALYYCARGESLGSPIYYYYGLDVWGQGTTVTVSS

SEQ ID NO: 331 - DNA, 24 bp, Artificial Sequence
  synthetic
ggattcaccctcagtaattttgtc

SEQ ID NO: 332 - protein, 8 aa, Artificial Sequence
  synthetic
GFTLSNFV

SEQ ID NO: 333 - DNA, 24 bp, Artificial Sequence
  synthetic
atattatatgatggaagtaataaa

SEQ ID NO: 334 - protein, 8 aa, Artificial Sequence
  synthetic
ILYDGSNK

SEQ ID NO: 335 - DNA, 54 bp, Artificial Sequence
  synthetic
gcgagaggagagtccttgggatcacctatctattattactacggtttggacgtc

SEQ ID NO: 336 - protein, 18 aa, Artificial Sequence
  synthetic
ARGESLGSPIYYYYGLDV

SEQ ID NO: 337 - DNA, 360 bp, Artificial Sequence
  synthetic
caggtgcagctgcaggagtcgggcccaggactggtgaagccttcggagaccctgtccctcacctgcattgtctctggtggctccatcagtggttacttctggaactggatccggcagcccccagggaagggacttgaatggattggttatatctattacagtgggaccaccatctacaacccctccctcaagagtcgattcaccatatcactagacacgtccaagaaccagttctccctaaagctgacctctgtgaccgctgcggacacggccgtatattactgtgcgagagagtcgtataatccctcgccgcgatattttgaccactggggccagggaaccctggtcaccgtctcctca

SEQ ID NO: 338 - protein, 120 aa, Artificial Sequence
  synthetic
QVQLQESGPGLVKPSETLSLTCIVSGGSISGYFWNWIRQPPGKGLEWIGYIYYSGTTIYNPSLKSRFTISLDTSKNQFSLKLTSVTAADTAVYYCARESYNPSPRYFDHWGQGTLVTVSS

SEQ ID NO: 339 - DNA, 24 bp, Artificial Sequence
  synthetic
ggtggctccatcagtggttacttc

SEQ ID NO: 340 - protein, 8 aa, Artificial Sequence
  synthetic
GGSISGYF

SEQ ID NO: 341 - DNA, 21 bp, Artificial Sequence
  synthetic
atctattacagtgggaccacc

SEQ ID NO: 342 - protein, 7 aa, Artificial Sequence
  synthetic
IYYSGTT

SEQ ID NO: 343 - DNA, 42 bp, Artificial Sequence
  synthetic
gcgagagagtcgtataatccctcgccgcgatattttgaccac

SEQ ID NO: 344 - protein, 14 aa, Artificial Sequence
  synthetic
ARESYNPSPRYFDH

SEQ ID NO: 345 - DNA, 375 bp, Artificial Sequence
  synthetic
caggtgcagctggtggagtctgggggaggcgtggtccagcctgggaggtccctgagactctcctgtgcagcgtctggattcagcttcagtagttatggcatgcactgggtccgccaggctccaggcaaggggctggagtggatggcagttatatggtatgctggaagtaataaattctatgcagactccgtgaagggccgattcaccatctccagagacaattccaagaacacgctgtatctgcaaatgaacagcctgacagccgaggacacggctgtatattactgtgcgagagggtcgagtctagcagctccagacctctacaagtacggaatggacgtctggggccaggggaccacggtcaccgtctcctca

SEQ ID NO: 346 - protein, 125 aa, Artificial Sequence
  synthetic
QVQLVESGGGVVQPGRSLRLSCAASGFSFSSYGMHWVRQAPGKGLEWMAVIWYAGSNKFYADSVKGRFTISRDNSKNTLYLQMNSLTAEDTAVYYCARGSSLAAPDLYKYGMDVWGQGTTVTVSS

SEQ ID NO: 347 - DNA, 24 bp, Artificial Sequence
  synthetic
ggattcagcttcagtagttatggc

SEQ ID NO: 348 - protein, 8 aa, Artificial Sequence
  synthetic
GFSFSSYG

SEQ ID NO: 349 - DNA, 24 bp, Artificial Sequence
  synthetic
atatggtatgctggaagtaataaa

SEQ ID NO: 350 - protein, 8 aa, Artificial Sequence
  synthetic
IWYAGSNK

SEQ ID NO: 351 - DNA, 54 bp, Artificial Sequence
  synthetic
gcgagagggtcgagtctagcagctccagacctctacaagtacggaatggacgtc

SEQ ID NO: 352 - protein, 18 aa, Artificial Sequence
  synthetic
ARGSSLAAPDLYKYGMDV

SEQ ID NO: 353 - DNA, 351 bp, Artificial Sequence
  synthetic
caggtgcagctgcaggagtcgggcccaggactggtgaagccttcggagaccctgtccctcacctgtactatctctggtggctccatcagtaattccttcttgacctggatccgacagcccccagggaagggactggagtggattggatatatctatcaccggggaaacactgattccaatccctccctcaagagtcgagtcaccatctcaacagacccgtccaagaatcagttctccctgaccctgcactctgtgaccgccgcagactcggccatatattactgtgcgcggggacaatttatggagtggtttgacttctggggccagggaaccctggtcaccgtctcctca

SEQ ID NO: 354 - protein, 117 aa, Artificial Sequence
  synthetic
QVQLQESGPGLVKPSETLSLTCTISGGSISNSFLTWIRQPPGKGLEWIGYIYHRGNTDSNPSLKSRVTISTDPSKNQFSLTLHSVTAADSAIYYCARGQFMEWFDFWGQGTLVTVSS

SEQ ID NO: 355 - DNA, 24 bp, Artificial Sequence
  synthetic
ggtggctccatcagtaattccttc

SEQ ID NO: 356 - protein, 8 aa, Artificial Sequence
  synthetic
GGSISNSF

SEQ ID NO: 357 - DNA, 21 bp, Artificial Sequence
  synthetic
atctatcaccggggaaacact

SEQ ID NO: 358 - protein, 7 aa, Artificial Sequence
  synthetic
IYHRGNT

SEQ ID NO: 359 - DNA, 33 bp, Artificial Sequence
  synthetic
gcgcggggacaatttatggagtggtttgacttc

SEQ ID NO: 360 - protein, 11 aa, Artificial Sequence
  synthetic
ARGQFMEWFDF

SEQ ID NO: 361 - DNA, 375 bp, Artificial Sequence
  synthetic
caggtgcagctggtggagtctgggggaggcgtggtccagcctgggaggtccctgagagtctcctgtgaagcgtctggattcaccctcagtagttatggcatgaactgggtccgccaggctccaggcaaggggctggagtgggtggcagttatatggtatgatggaagtaataaatactattcagactccgtgaagggccgattcaccatctccagagacaattccaagaacacgctgtatctgcaaatgaacggcctgagagacgatgacacggctgtgtattactgtgcgagaggggagcagctcggctctcatgtctattattactatggaatggacgtctggggccaagggaccacggtcaccgtctcctca

SEQ ID NO: 362 - protein, 125 aa, Artificial Sequence
  synthetic
QVQLVESGGGVVQPGRSLRVSCEASGFTLSSYGMNWVRQAPGKGLEWVAVIWYDGSNKYYSDSVKGRFTISRDNSKNTLYLQMNGLRDDDTAVYYCARGEQLGSHVYYYYGMDVWGQGTTVTVSS

SEQ ID NO: 363 - DNA, 24 bp, Artificial Sequence
  synthetic
ggattcaccctcagtagttatggc

SEQ ID NO: 364 - protein, 8 aa, Artificial Sequence
  synthetic
GFTLSSYG

SEQ ID NO: 365 - DNA, 24 bp, Artificial Sequence
  synthetic
atatggtatgatggaagtaataaa

SEQ ID NO: 366 - protein, 8 aa, Artificial Sequence
  synthetic
IWYDGSNK

SEQ ID NO: 367 - DNA, 54 bp, Artificial Sequence
  synthetic
gcgagaggggagcagctcggctctcatgtctattattactatggaatggacgtc

SEQ ID NO: 368 - protein, 18 aa, Artificial Sequence
  synthetic
ARGEQLGSHVYYYYGMDV

SEQ ID NO: 369 - DNA, 375 bp, Artificial Sequence
  synthetic
caggtgcagctggtggagtctgggggaggcgtggtccagcctgggaagtccctgagactctcctgtgcagcgtctggattcaccttcagtaactatgtcatgcactgggtccgccagactccaggcaaggggctggagtgggtggcgattattttatttcctggaagtaataaatactatgtagactccgtgcagggccgattcaccatctccagagacaattccaagaacacgctgtctctgcaaatgaacagcctgagagccgaagacacggctgtatattactgtgcgaggggctcgagtttgacagctcttgactactactactacggtctggacgtctggggccaagggaccacggtcaccgtctcctca

SEQ ID NO: 370 - protein, 125 aa, Artificial Sequence
  synthetic
QVQLVESGGGVVQPGKSLRLSCAASGFTFSNYVMHWVRQTPGKGLEWVAIILFPGSNKYYVDSVQGRFTISRDNSKNTLSLQMNSLRAEDTAVYYCARGSSLTALDYYYYGLDVWGQGTTVTVSS

SEQ ID NO: 371 - DNA, 24 bp, Artificial Sequence
  synthetic
ggattcaccttcagtaactatgtc

SEQ ID NO: 372 - protein, 8 aa, Artificial Sequence
  synthetic
GFTFSNYV

SEQ ID NO: 373 - DNA, 24 bp, Artificial Sequence
  synthetic
attttatttcctggaagtaataaa

SEQ ID NO: 374 - protein, 8 aa, Artificial Sequence
  synthetic
ILFPGSNK

SEQ ID NO: 375 - DNA, 54 bp, Artificial Sequence
  synthetic
gcgaggggctcgagtttgacagctcttgactactactactacggtctggacgtc

SEQ ID NO: 376 - protein, 18 aa, Artificial Sequence
  synthetic
ARGSSLTALDYYYYGLDV

SEQ ID NO: 377 - DNA, 375 bp, Artificial Sequence
  synthetic
caggtgcagctggtggagtctgggggaggcgtggtccagcctgggaggtccctgagactctcctgtgcagcgtctggattcaccttcagtaactatgtcatgcactgggtccgccaggctccaggcaaggggctggagtgggtggcaattatatggtatgatggaactaatgaagactatgcagactccgtgaaggtccgattcaccatctccagagacatttccaagaacacgctgtatctgcaaatgaacagcctgagagccgaggacacggctgtatattactgtgcgagagattggtttgattgtagtagtaccagctgctataggtacttcgatctctggggccgtggcaccctggtcactgtctcctca

SEQ ID NO: 378 - protein, 125 aa, Artificial Sequence
  synthetic
QVQLVESGGGVVQPGRSLRLSCAASGFTFSNYVMHWVRQAPGKGLEWVAIIWYDGTNEDYADSVKVRFTISRDISKNTLYLQMNSLRAEDTAVYYCARDWFDCSSTSCYRYFDLWGRGTLVTVSS

SEQ ID NO: 379 - DNA, 24 bp, Artificial Sequence
  synthetic
ggattcaccttcagtaactatgtc

SEQ ID NO: 380 - protein, 8 aa, Artificial Sequence
  synthetic
GFTFSNYV

SEQ ID NO: 381 - DNA, 24 bp, Artificial Sequence
  synthetic
atatggtatgatggaactaatgaa

SEQ ID NO: 382 - protein, 8 aa, Artificial Sequence
  synthetic
IWYDGTNE

SEQ ID NO: 383 - DNA, 54 bp, Artificial Sequence
  synthetic
gcgagagattggtttgattgtagtagtaccagctgctataggtacttcgatctc

SEQ ID NO: 384 - protein, 18 aa, Artificial Sequence
  synthetic
ARDWFDCSSTSCYRYFDL

SEQ ID NO: 385 - DNA, 375 bp, Artificial Sequence
  synthetic
caggtgcagctggtggagtctgggggaggcgtggtccagcctgggaggtccctgagactctcctgtgcagcgtctggattcaccttcagtaataataacatgcactgggtccgccaggctccaggcaaggggctggagtgggtggcagttatatggtatgatggaagtaataaagattatgtagactccgtgaagggccgattcaccatctccagagacaattccaagaacacgctgtatctgcaaatgaacagtttgagagccgaggatacggctgtgtattattgtgcgagatttgtagtagcgccagctacgtactcctactactacattatagacgtctggggccaagggaccacggtcaccgtctcctca

SEQ ID NO: 386 - protein, 125 aa, Artificial Sequence
  synthetic
QVQLVESGGGVVQPGRSLRLSCAASGFTFSNNNMHWVRQAPGKGLEWVAVIWYDGSNKDYVDSVKGRFTISRDNSKNTLYLQMNSLRAEDTAVYYCARFVVAPATYSYYYIIDVWGQGTTVTVSS

SEQ ID NO: 387 - DNA, 24 bp, Artificial Sequence
  synthetic
ggattcaccttcagtaataataac

SEQ ID NO: 388 - protein, 8 aa, Artificial Sequence
  synthetic
GFTFSNNN

SEQ ID NO: 389 - DNA, 24 bp, Artificial Sequence
  synthetic
atatggtatgatggaagtaataaa

SEQ ID NO: 390 - protein, 8 aa, Artificial Sequence
  synthetic
IWYDGSNK

SEQ ID NO: 391 - DNA, 54 bp, Artificial Sequence
  synthetic
gcgagatttgtagtagcgccagctacgtactcctactactacattatagacgtc

SEQ ID NO: 392 - protein, 18 aa, Artificial Sequence
  synthetic
ARFVVAPATYSYYYIIDV

SEQ ID NO: 393 - DNA, 378 bp, Artificial Sequence
  synthetic
caggtgcagctggtggagtctgggggaggcgtggtccagcctgggaggtccctgagactctcctgtgcagcctctggatttaccttcagtacctatggcatgcactgggtccgccaggctccaggcaaggggctggagtgggtggcagttatttcatatgatggaagaattaaatactatgaagactccgtgaagggccgattcatcatatccagagacaactccaagaacacactgtatctgcaagtgaacaccctgagagctgaggacacggctgtgtattactgtgcgaaagagaggagatattgtagtgatactaatacctgctctgatgtttttgatgtctggggccaggggacaatggtcaccgtctcttca

SEQ ID NO: 394 - protein, 126 aa, Artificial Sequence
  synthetic
QVQLVESGGGVVQPGRSLRLSCAASGFTFSTYGMHWVRQAPGKGLEWVAVISYDGRIKYYEDSVKGRFIISRDNSKNTLYLQVNTLRAEDTAVYYCAKERRYCSDTNTCSDVFDVWGQGTMVTVSS

SEQ ID NO: 395 - DNA, 24 bp, Artificial Sequence
  synthetic
ggatttaccttcagtacctatggc

SEQ ID NO: 396 - protein, 8 aa, Artificial Sequence
  synthetic
GFTFSTYG

SEQ ID NO: 397 - DNA, 24 bp, Artificial Sequence
  synthetic
atttcatatgatggaagaattaaa

SEQ ID NO: 398 - protein, 8 aa, Artificial Sequence
  synthetic
ISYDGRIK

SEQ ID NO: 399 - DNA, 57 bp, Artificial Sequence
  synthetic
gcgaaagagaggagatattgtagtgatactaatacctgctctgatgtttttgatgtc

SEQ ID NO: 400 - protein, 19 aa, Artificial Sequence
  synthetic
AKERRYCSDTNTCSDVFDV

SEQ ID NO: 401 - DNA, 324 bp, Artificial Sequence
  synthetic
gacatccagatgacccagtctccatcctccctgtctgcatctgtaggagacagagtcaccatcacttgccgggcaagtcagagcattagcagctatttaaattggtatcagcagaaaccagggaaagcccctaagctcctgatctatgctgcatccagtttgcaaagtggggtcccgtcaaggttcagtggcagtggatctgggacagatttcactctcaccatcagcagtctgcaacctgaagattttgcaacttactactgtcaacagagttacagtacccctccgatcaccttcggccaagggacacgactggagattaaa

SEQ ID NO: 402 - protein, 108 aa, Artificial Sequence
  synthetic
DIQMTQSPSSLSASVGDRVTITCRASQSISSYLNWYQQKPGKAPKLLIYAASSLQSGVPSRFSGSGSGTDFTLTISSLQPEDFATYYCQQSYSTPPITFGQGTRLEIK

SEQ ID NO: 403 - DNA, 18 bp, Artificial Sequence
  synthetic
cagagcattagcagctat

SEQ ID NO: 404 - protein, 6 aa, Artificial Sequence
  synthetic
QSISSY

SEQ ID NO: 405 - DNA, 9 bp, Artificial Sequence
  synthetic
gctgcatcc

SEQ ID NO: 406 - protein, 3 aa, Artificial Sequence
  synthetic
AAS

SEQ ID NO: 407 - DNA, 30 bp, Artificial Sequence
  synthetic
caacagagttacagtacccctccgatcacc

SEQ ID NO: 408 - protein, 10 aa, Artificial Sequence
  synthetic
QQSYSTPPIT

SEQ ID NO: 409 - protein, 194 aa, Artificial Sequence
  synthetic
MHRPRRRGTRPPPLALLAALLLAARGADAQRPTGGPGCGPGRLLLGTGTDARCCRVHTTRCCRDYPGEECCSEWDCMCVQPEFHCGDPCCTTCRHHPCPPGQGVQSQGKFSFGFQCIDCASGTFSGGHEGHCKPWTDCTQFGFLTVFPGNKTHNAVCVPGSPPAEPEQKLISEEDLGGEQKLISEEDLHHHHHH

SEQ ID NO: 410 - protein, 399 aa, Artificial Sequence
  synthetic
MHRPRRRGTRPPPLALLAALLLAARGADAQRPTGGPGCGPGRLLLGTGTDARCCRVHTTRCCRDYPGEECCSEWDCMCVQPEFHCGDPCCTTCRHHPCPPGQGVQSQGKFSFGFQCIDCASGTFSGGHEGHCKPWTDCTQFGFLTVFPGNKTHNAVCVPGSPPAEPEPRGPTIKPCPPCKCPAPNLLGGPSVFIFPPKIKDVLMISLSPIVTCVVVDVSEDDPDVQISWFVNNVEVHTAQTQTHREDYNSTLRVVSALPIQHQDWMSGKEFKCKVNNKDLPAPIERTISKPKGSVRAPQVYVLPPPEEEMTKKQVTLTCMVTDFMPEDIYVEWTNNGKTELNYKNTEPVLDSDGSYFMYSKLRVEKKNWVERNSYSCSVVHEGLHNHHTTKSFSRTPGK

SEQ ID NO: 411 - protein, 393 aa, Artificial Sequence
  synthetic
MHRPRRRGTRPPPLALLAALLLAARGADAQRPTGGPGCGPGRLLLGTGTDARCCRVHTTRCCRDYPGEECCSEWDCMCVQPEFHCGDPCCTTCRHHPCPPGQGVQSQGKFSFGFQCIDCASGTFSGGHEGHCKPWTDCTQFGFLTVFPGNKTHNAVCVPGSPPAEPDKTHTCPPCPAPELLGGPSVFLFPPKPKDTLMISRTPEVTCVVVDVSHEDPEVKFNWYVDGVEVHNAKTKPREEQYNSTYRVVSVLTVLHQDWLNGKEYKCKVSNKALPAPIEKTISKAKGQPREPQVYTLPPSRDELTKNQVSLTCLVKGFYPSDIAVEWESNGQPENNYKTTPPVLDSDGSFFLYSKLTVDKSRWQQGNVFSCSVMHEALHNHYTQKSLSLSPGK

SEQ ID NO: 412 - protein, 194 aa, Artificial Sequence
  synthetic
MHRPRRRGTRPPPLALLAALLLAARGADAQRPTGGPGCGPGRLLLGTGKDARCCRVHPTRCCRDYQGEECCSEWDCVCVQPEFHCGNPCCTTCQHHPCPSGQGVQPQGKFSFGFRCVDCALGTFSRGHDGHCKPWTDCTQFGFLTVFPGNKTHNAVCVPGSPPAEPEQKLISEEDLGGEQKLISEEDLHHHHHH

SEQ ID NO: 413 - protein, 241 aa, Artificial Sequence
  synthetic
MAQHGAMGAFRALCGLALLCALSLGQRPTGGPGCGPGRLLLGTGTDARCCRVHTTRCCRDYPGEECCSEWDCMCVQPEFHCGDPCCTTCRHHPCPPGQGVQSQGKFSFGFQCIDCASGTFSGGHEGHCKPWTDCTQFGFLTVFPGNKTHNAVCVPGSPPAEPLGWLTVVLLAVAACVLLLTSAQLGLHIWQLRSQCMWPRETQLLLEVPPSTEDARSCQFPEEERGERSAEEKGRLGDLWV